European Patent Application EP 4 491 725 A1, published January 15, 2025. Title: Method for ecological survey on fishes in freshwater environment. Applicant: KAO CORPORATION. The sequence listing filed with the application follows.

SEQUENCE LISTING (3 sequences)

SEQ ID NO: 1 - DNA, 20 bp, synthetic construct
  misc_feature 1..20: note = Oligonucleotide primer
  source 1..20: mol_type = other DNA
tttgcctacgccattctacg

SEQ ID NO: 2 - DNA, 23 bp, synthetic construct
  misc_feature 1..23: note = Oligonucleotide primer
  source 1..23: mol_type = other DNA
ggcttcgttgtttagaggtgtga

SEQ ID NO: 3 - DNA, 24 bp, synthetic construct
  misc_feature 1..24: note = Oligonucleotide probe
  source 1..24: mol_type = other DNA
ttagcctctattctagtactattc